European Patent Specification EP 3 737 357 B1, published March 1, 2023. Title: Anionic nanocomplexes for nucleic acid delivery. Applicant: UCL Business PLC. The sequence listing filed with the application follows.

SEQUENCE LISTING (16 sequences)

SEQ ID NO: 1 - protein, 4 aa, Artificial Sequence
  cleavable portion of the spacer element peptide B
RVRR

SEQ ID NO: 2 - protein, 9 aa, Artificial Sequence
  Receptor binding sequence of the cell surface receptor binding component C
  MISC_FEATURE (2)..(7): The residue at each of these positions can be P or Q
LPPPPPPHK

SEQ ID NO: 3 - protein, 16 aa, Artificial Sequence
  Oligolysine polycationic nucleic acid binding component
KKKKKKKKKKKKKKKK

SEQ ID NO: 4 - protein, 5 aa, Artificial Sequence
  A linker sequence of the spacer element peptide B
  MOD_RES (1)..(1): 6-amino hexanoic acid
  MOD_RES (3)..(3): 6-amino hexanoic acid
XSXGG

SEQ ID NO: 5 - protein, 5 aa, Artificial Sequence
  A linker sequence of the spacer element peptide B
  MOD_RES (1)..(1): 6-aminohexanoic acid
  MOD_RES (3)..(3): 6-aminohexanoic acid
XSXGA

SEQ ID NO: 6 - protein, 6 aa, Artificial Sequence
  A cleavable sequence and a linker sequence in the spacer element peptide B
RVRRGA

SEQ ID NO: 7 - protein, 6 aa, Artificial Sequence
  A cleavable sequence and a linker sequence in the spacer element peptide B
RVRRGC

SEQ ID NO: 8 - protein, 7 aa, Artificial Sequence
  A cleavable sequence and a linker sequence in the spacer element peptide B
  MOD_RES (5)..(5): 6-amino hexanoic acid
  MOD_RES (7)..(7): 6-amino hexanoic acid
RVRRXSX

SEQ ID NO: 9 - protein, 9 aa, Artificial Sequence
  A cleavable sequence and a linker sequence in the spacer element peptide B
  MOD_RES (5)..(5): 6-amino hexanoic acid
  MOD_RES (7)..(7): 6-amino hexanoic acid
RVRRXSXGA

SEQ ID NO: 10 - protein, 9 aa, Artificial Sequence
  A cleavable sequence and a linker sequence in the spacer element peptide B
  MOD_RES (5)..(5): 6-amino hexanoic acid
  MOD_RES (7)..(7): 6-amino hexanoic acid
RVRRXSXGC

SEQ ID NO: 11 - protein, 7 aa, Artificial Sequence
  Component of the cell surface receptor binding component C
YGLPHKF

SEQ ID NO: 12 - protein, 10 aa, Artificial Sequence
  Component of the cell surface receptor binding component C
CYGLPHKFCG

SEQ ID NO: 13 - protein, 35 aa, Artificial Sequence
  Peptide 35 for use in accordance with the invention
  MOD_RES (21)..(21): 6-amino hexanoic acid
  MOD_RES (23)..(23): 6-amino hexanoic acid
KKKKKKKKKKKKKKKKRVRRXSXGACYGLPHKFCG

SEQ ID NO: 14 - protein, 32 aa, Artificial Sequence
  Peptide 32 for use in accordance with the invention
KKKKKKKKKKKKKKKKRVRRGACYGLPHKFCG

SEQ ID NO: 15 - protein, 29 aa, Artificial Sequence
  Peptide ME27 for use in accordance with the invention
KKKKKKKKKKKKKKKKRVRRGACRGDCLG

SEQ ID NO: 16 - protein, 28 aa, Artificial Sequence
  Peptide Y for use in accordance with the invention
KKKKKKKKKKKKKKKKGACYGLPHKFCG